European Patent Specification EP 3 262 061 B1, published July 12, 2023. Title: Peptides and uses thereof. Applicant: FUNDACIÓ CENTRE DE REGULACIÓ GENÒMICA (CRG) INSTITUCIO CATALANA DE RECERCA I ESTUDIS AVANCATS. The sequence listing filed with the application follows.

SEQUENCE LISTING (12 sequences)

SEQ ID NO: 1 - protein, 28 aa, Mycoplasma pneumoniae
  SOURCE 1..28: /mol_type="protein" /organism="Mycoplasma pneumoniae"
MKSKLKLKRYLLFLPLLPLGTLSLANTY

SEQ ID NO: 2 - protein, 28 aa, Mycoplasma pneumoniae
  SOURCE 1..28: /mol_type="protein" /organism="Mycoplasma pneumoniae"
MKLKLKFLLISLLGSSLLLSACSSAATQ

SEQ ID NO: 3 - protein, 38 aa, Mycoplasma pneumoniae
  SOURCE 1..38: /mol_type="protein" /organism="Mycoplasma pneumoniae"
MKLNFKIKDKKTLKRLKKGGFWALGLFGAAINAFSAVL

SEQ ID NO: 4 - protein, 25 aa, Mycoplasma pneumoniae
  SOURCE 1..25: /mol_type="protein" /note="Mpn-200" /organism="Mycoplasma pneumoniae"
MKFKYGAIVFSGLLGVSAILAACGT

SEQ ID NO: 5 - protein, 31 aa, Mycoplasma pneumoniae
  SOURCE 1..31: /mol_type="protein" /note="Mpn-213" /organism="Mycoplasma pneumoniae"
MKLSAIISLSVAGTVGTTAVVVPTTITLVNK

SEQ ID NO: 6 - protein, 31 aa, Mycoplasma pneumoniae
  SOURCE 1..31: /mol_type="protein" /note="Mpn-489" /organism="Mycoplasma pneumoniae"
MGYKLKRWPLVAFTFTGIGLGVVLAACSALN

SEQ ID NO: 7 - DNA, 84 bp, artificial sequences
  source 1..84: /mol_type="DNA" /note="optimized sequence coding peptide Mpn142" /organism="artificial sequences"
atgaagtccaagttgaaactcaaacgctatttactctttctccccttgttaccactcggtaccttgagtttagctaacacttac

SEQ ID NO: 8 - DNA, 84 bp, Mycoplasma pneumoniae
  source 1..84: /mol_type="DNA" /note="Mpn-142" /organism="Mycoplasma pneumoniae"
atgaaatcgaagctaaagttaaaacgttatttactgtttttaccacttttaccgctagggacgttgtcactagccaacacctac

SEQ ID NO: 9 - DNA, 84 bp, Mycoplasma pneumoniae
  source 1..84: /mol_type="DNA" /note="Mpn-645" /organism="Mycoplasma pneumoniae"
atgaaactgaaacttaaatttctattaatttctcttttaggttctagtttgttgttaagcgcttgttcttcagcagctactcaa

SEQ ID NO: 10 - DNA, 75 bp, Mycoplasma pneumoniae
  source 1..75: /mol_type="DNA" /note="Mpn-200" /organism="Mycoplasma pneumoniae"
atgaaatttaagtatggtgccattgttttcagtggtcttttaggagtctctgccattttagctgcttgtggtaca

SEQ ID NO: 11 - DNA, 93 bp, Mycoplasma pneumoniae
  source 1..93: /mol_type="DNA" /note="Mpn-213" /organism="Mycoplasma pneumoniae"
atgaagcttagtgctattatctccctatcagtcgctggtactgtgggaacaactgcggtggtagtacctacaactataacgcttgtaaataag

SEQ ID NO: 12 - DNA, 150 bp, Escherichia coli
  source 1..150: /mol_type="DNA" /organism="Escherichia coli"
gaagaccttttgtgctaacgccagtttggcaaatcaagttctgattttgcaattattttgctccatatgaattacactactccaagaattataagcctctctacagctttatctcaaacttatgtaaaattagagacgtaattcaaacac